European Patent Application EP 4 563 528 A1, published June 4, 2025. Title: Mesoporous silica nanoparticles and their use in the uptake of immunoglobulins. Applicant: SERVICIO ANDALUZ DE SALUD. Application ES. The sequence listing filed with the application follows.

SEQUENCE LISTING (2 sequences)

SEQ ID NO: 1 - protein, 185 aa, synthetic construct
MKGETTTEAVDAATAEKVFKQYANDNGVDGEWTYDDATKTFTVTEKPEVIDASELTPAVTTYKLVINGKTLKGETTTEAVDAATAEKVFKQYANDNGVDGEWTYDDATKTFTVTEKPEVIDASELTPAVTTYKLVINGKTLKGETTTKAVDAETAEKAFKQYANDNGVDGVWTYDDATKTFTVTE

SEQ ID NO: 2 - protein, 71 aa, Staphylococcus aureus
LNMPNLNADQRNGFIQSLKDDPSQSANLLSEAKKLNESQAPKADNKFNKEQQNAFYEILHLPNLNEEQRNG